European Patent Specification EP 4 022 089 B1, published August 21, 2024. Title: METHODS FOR IDENTIFYING A COMPANION ANIMAL AT RISK OF CALCIUM OXALATE STONE FORMATION AND TREATMENTS AND COMPOSITIONS FOR REDUCING THE RISK. Applicant: Hill's Pet Nutrition, Inc. The sequence listing filed with the application follows.

SEQUENCE LISTING (1 sequence)

SEQ ID NO: 1 - DNA, 201 bp, Felis catus
atatgttagtatctctacatgtgggagaaccagatgtcaggttcatgtatgatacagcaggaagaacacagcacggcctttgaagtattcctgtttatagraataattctttcatatgcaggtacgtgtgtgtgtgtgtgtgtgtgtgtgtgtgtgtgtgtgtgtattttataaaggtagctactccttattcatagatat